European Patent Specification EP 4 117 667 B1, published December 18, 2024. Title: SEQUENTIAL TREATMENT OF CANCERS USING 6-THIO-dG, CHECKPOINT INHIBITORS AND RADIATION THERAPY. Applicant: The Board of Regents of the University of Texas System. Application Unknown. The sequence listing filed with the application follows.

SEQUENCE LISTING (10 sequences)

SEQ ID NO: 1 - DNA, 20 bp, Artificial sequence
  Synthetic oligo
cacctagcctcgcacgaact

SEQ ID NO: 2 - DNA, 20 bp, Artificial sequence
  Synthetic oligo
cgcaaaggggggctcgatcg

SEQ ID NO: 3 - DNA, 20 bp, Artificial sequence
  Synthetic oligo
cgccacactccacggaagca

SEQ ID NO: 4 - DNA, 20 bp, Artificial sequence
  Synthetic oligo
cggggcattccggataggcc

SEQ ID NO: 5 - DNA, 22 bp, Artificial sequence
  Synthetic oligo
accgattggatggtttagtgag

SEQ ID NO: 6 - DNA, 22 bp, Artificial sequence
  Synthetic oligo
cctacggaaaccttgttacgac

SEQ ID NO: 7 - DNA, 19 bp, Artificial sequence
  Synthetic oligo
atgagtggtggttgcaggc

SEQ ID NO: 8 - DNA, 25 bp, Artificial sequence
  Synthetic oligo
tgacctttcaaatgcagtagattca

SEQ ID NO: 9 - DNA, 20 bp, Artificial sequence
  Synthetic oligo
catcaagaaggtggtgaagc

SEQ ID NO: 10 - DNA, 20 bp, Artificial sequence
  Synthetic oligo
cctgttgctgtagccgtatt